European Patent Application EP 4 647 440 A1, published November 12, 2025. Title: Immunogenic TROP2 peptides. Applicant: Aston Sci., Co. Ltd. The sequence listing filed with the application follows.

SEQUENCE LISTING (27 sequences)

SEQ ID NO: 1 - protein, 323 aa, Homo sapiens
MARGPGLAPPPLRLPLLLLVLAAVTGHTAAQDNCTCPTNKMTVCSPDGPGGRCQCRALGSGMAVDCSTLTSKCLLLKARMSAPKNARTLVRPSEHALVDNDGLYDPDCDPEGRFKARQCNQTSVCWCVNSVGVRRTDKGDLSLRCDELVRTHHILIDLRHRPTAGAFNHSDLDAELRRLFRERYRLHPKFVAAVHYEQPTIQIELRQNTSQKAAGDVDIGDAAYYFERDIKGESLFQGRGGLDLRVRGEPLQVERTLIYYLDEIPPKFSMKRLTAGLIAVIVVVVVALVAGMAVLVITNRRKSGKYKKVEIKELGELRKEPSL

SEQ ID NO: 2 - protein, 15 aa, synthetic construct
PPPLRLPLLLLVLAA

SEQ ID NO: 3 - protein, 22 aa, synthetic construct
PLRLPLLLLVLAAVTGHTAAQD

SEQ ID NO: 4 - protein, 15 aa, synthetic construct
PLLLLVLAAVTGHTA

SEQ ID NO: 5 - protein, 15 aa, synthetic construct
LVLAAVTGHTAAQDN

SEQ ID NO: 6 - protein, 15 aa, synthetic construct
STLTSKCLLLKARMS

SEQ ID NO: 7 - protein, 15 aa, synthetic construct
TSKCLLLKARMSAPK

SEQ ID NO: 8 - protein, 15 aa, synthetic construct
SKCLLLKARMSAPKN

SEQ ID NO: 9 - protein, 15 aa, synthetic construct
CLLLKARMSAPKNAR

SEQ ID NO: 10 - protein, 15 aa, synthetic construct
LVRPSEHALVDNDGL

SEQ ID NO: 11 - protein, 27 aa, synthetic construct
SLRCDELVRTHHILIDLRHRPTAGAFN

SEQ ID NO: 12 - protein, 15 aa, synthetic construct
DELVRTHHILIDLRH

SEQ ID NO: 13 - protein, 15 aa, synthetic construct
HHILIDLRHRPTAGA

SEQ ID NO: 14 - protein, 15 aa, synthetic construct
LFRERYRLHPKFVAA

SEQ ID NO: 15 - protein, 15 aa, synthetic construct
RERYRLHPKFVAAVH

SEQ ID NO: 16 - protein, 15 aa, synthetic construct
ERYRLHPKFVAAVHY

SEQ ID NO: 17 - protein, 15 aa, synthetic construct
ELRQNTSQKAAGDVD

SEQ ID NO: 18 - protein, 15 aa, synthetic construct
RGEPLQVERTLIYYL

SEQ ID NO: 19 - protein, 15 aa, synthetic construct
EPLQVERTLIYYLDE

SEQ ID NO: 20 - protein, 15 aa, synthetic construct
TLIYYLDEIPPKFSM

SEQ ID NO: 21 - protein, 15 aa, synthetic construct
IPPKFSMKRLTAGLI

SEQ ID NO: 22 - protein, 17 aa, synthetic construct
PKFSMKRLTAGLIAVIV

SEQ ID NO: 23 - protein, 15 aa, synthetic construct
KFSMKRLTAGLIAVI

SEQ ID NO: 24 - protein, 34 aa, synthetic construct
AGLIAVIVVVVVALVAGMAVLVITNRRKSGKYKK

SEQ ID NO: 25 - protein, 15 aa, synthetic construct
VVVVVALVAGMAVLV

SEQ ID NO: 26 - protein, 15 aa, synthetic construct
GMAVLVITNRRKSGK

SEQ ID NO: 27 - protein, 15 aa, synthetic construct
LVITNRRKSGKYKKV